European Patent Specification EP 3 603 384 B1, published April 17, 2024. Title: Plant resistant to a pathogen. Applicant: Syngenta Participations AG. The sequence listing filed with the application follows.

SEQUENCE LISTING (16 sequences)

SEQ ID NO: 1 - DNA, 19 bp, Artificial Sequence
  Forward primer for SSR-Marker NL0918
ccattaatccaaaggcaac

SEQ ID NO: 2 - DNA, 19 bp, Artificial sequence
  Revers pirmer for SSR-Marker NL0918
ccagtgaaggaagcaaaag

SEQ ID NO: 3 - DNA, 19 bp, Artificial sequence
  Forward primer for SSR-Marker NL0920
gatggaaccactttggatg

SEQ ID NO: 4 - DNA, 19 bp, Artificial sequence
  Revers primer for SSR-Marker NL0920
cctgcaacaagatgtgatg

SEQ ID NO: 5 - DNA, 21 bp, Artificial sequence
  Forward primer for SNP 272 from SSR NL0918
attccacttgcatttatctgg

SEQ ID NO: 6 - DNA, 21 bp, Artificial sequence
  Revers primer for SNP 272 from SSR NL0918
ccccatttgatatttcttgat

SEQ ID NO: 7 - DNA, 23 bp, Artificial sequence
  Forward primer for SNP 430 from SSR NL0920
tggaaagatgtgaaatccatata

SEQ ID NO: 8 - DNA, 25 bp, Artificial sequence
  Revers primer for SNP 430 from SSR NL0920
gagtttcagctaagtgtaatcaaat

SEQ ID NO: 9 - DNA, 26 bp, Artificial sequence
  Forward primer for SNP 305 from SSR NL0920
tgtgctcagttgatataagaattagt

SEQ ID NO: 10 - DNA, 26 bp, Artificial sequence
  Revers primer for SNP 305 from SSR NL0920
ccaaattggataaaataaacctacac

SEQ ID NO: 11 - DNA, 15 bp, Artificial sequence
  Probe molecule for SNP 272 (R)
ctacactcccacaat

SEQ ID NO: 12 - DNA, 13 bp, Artificial sequence
  Probe molecule for SNP 272 (S)
actccaacaatct

SEQ ID NO: 13 - DNA, 13 bp, Artificial sequence
  Probe molecule for SNP 430 (R)
tgcagggagttaa

SEQ ID NO: 14 - DNA, 14 bp, Artificial sequence
  Probe molecule for SNP 430 (S)
tgcagagagttaac

SEQ ID NO: 15 - DNA, 14 bp, Artificial sequence
  Probe molecule for SNP 305 (R)
aagcatgtttcttg

SEQ ID NO: 16 - DNA, 13 bp, Artificial sequence
  Probe molecule for SNP 305 (S)
agcaggtttcttg